European Patent Application EP 4 656 723 A1, published December 3, 2025. Title: Luciferace mutant. Applicant: Kikkoman Corporation. The sequence listing filed with the application follows.

SEQUENCE LISTING (74 sequences)

SEQ ID NO: 1 - protein, 548 aa, Luciola lateralis
MENMENDENIVYGPEPFYPIEEGSAGAQLRKYMDRYAKLGAIAFTNALTGVDYTYAEYLEKSCCLGEALKNYGLVVDGRIALCSENCEEFFIPVLAGLFIGVGVAPTNEIYTLRELVHSLGISKPTIVFSSKKGLDKVITVQKTVTAIKTIVILDSKVDYRGYQSMDNFIKKNTPQGFKGSSFKTVEVNRKEQVALIMNSSGSTGLPKGVQLTHENAVTRFSHARDPIYGNQVSPGTAILTVVPFHHGFGMFTTLGYLTCGFRIVMLTKFDEETFLKTLQDYKCSSVILVPTLFAILNRSELLDKYDLSNLVEIASGGAPLSKEIGEAVARRFNLPGVRQGYGLTETTSAIIITPEGDDKPGASGKVVPLFKAKVIDLDTKKTLGPNRRGEVCVKGPMLMKGYVDNPEATREIIDEEGWLHTGDIGYYDEEKHFFIVDRLKSLIKYKGYQVPPAELESVLLQHPNIFDAGVAGVPDPIAGELPGAVVVLEKGKSMTEKEVMDYVASQVSNAKRLRGGVRFVDEVPKGLTGKIDGKAIREILKKPVAKM

SEQ ID NO: 2 - protein, 548 aa, Luciola lateralis
MENMENDENIVYGPEPFYPIEEGSAGAQLRKYMDRYAKLGAIAFTNALTGVDYTYAEYLEKSCCLGEALKNYGLVVDGRIALCSENCEEFFIPVLAGLFIGVGVAPTNEIYTLRELVHSLGISKPTIVFSSKKGLDKVITVQKTVTAIKTIVILDSKVDYRGYQSMDNFIKKNTPQGFKGSSFKTVEVNRKEQVALIMNSSGSTGLPKGVQLTHENLVTRFSHARDPIYGNQVSPGTAILTVVPFHHGFGMFTTLGYLTCGFRIVMLTKFDEETFLKTLQDYKCSSVILVPTLFAILNRSELLDKYDLSNLVEIASGGAPLSKEIGEAVARRFNLPGVRQGYGLTETTSAIIITPEGDDKPGASGKVVPLFKAKVIDLDTKKTLGPNRRGEVLVKGPMLMKGYVDNPEATREIIDEEGWLHTGDIGYYDEEKHFFIVDRLKSLIKYKGYQVPPAELESVLLQHPNIFDAGVAGVPDPIAGELPGAVVVLKKGKSMTEKEVMDYVASQVSNAKRLRGGVRFVDEVPKGLTGKIDGKAIREILKKPVAKM

SEQ ID NO: 3 - DNA, 1647 bp, Luciola lateralis
  source 1..1647: mol_type = other DNA
atggaaaacatggagaacgatgaaaatattgtgtatggtcctgaaccattttaccctattgaagagggatctgctggagcacaattgcgcaagtatatggatcgatatgcaaaacttggagcaattgcttttactaacgcacttaccggtgtcgattatacgtacgccgaatacttagaaaaatcatgctgtctaggagaggctttaaagaattatggtttggttgttgatggaagaattgcgttatgcagtgaaaactgtgaagagttctttattcctgtattagccggtttatttataggtgtcggtgtggctccaactaatgagatttacactctacgtgaattggttcacagtttaggcatctctaagccaacaattgtatttagttctaaaaaaggattagataaagttataactgtacaaaaaacggtaactgctattaaaaccattgttatattggacagcaaagtggattatagaggttatcaatccatggacaactttattaaaaaaaacactccacaaggtttcaaaggatcaagttttaaaactgtagaagttaaccgcaaagaacaagttgctcttataatgaactcttcgggttcaaccggtttgccaaaaggtgtgcaacttactcatgaaaatttggtcacgcgtttttctcacgctagagatccaatttatggaaaccaagtttcaccaggcacggctattttaactgtagtaccattccatcatggttttggtatgtttactactttaggctatctaacttgtggttttcgtattgtcatgttaacgaaatttgacgaagagacttttttaaaaacactgcaagattacaaatgttcaagcgttattcttgtaccgactttgtttgcaattcttaatagaagtgaattactcgataaatatgatttatcaaatttagttgaaattgcatctggcggagcacctttatctaaagaaattggtgaagctgttgctagacgttttaatttaccgggtgttcgtcaaggctatggtttaacagaaacaacctctgcaattattatcacaccggaaggcgatgataaaccaggtgcttctggcaaagttgtgccattatttaaagcaaaagttatcgatcttgatactaaaaaaactttgggcccgaacagacgtggagaagttctggtaaagggtcctatgcttatgaaaggttatgtagataatccagaagcaacaagagaaatcatagatgaagaaggttggttgcacacaggagatattgggtattacgatgaagaaaaacatttctttatcgtggatcgtttgaagtctttaatcaaatacaaaggatatcaagtaccacctgctgaattagaatctgttcttttgcaacatccaaatatttttgatgccggcgttgctggcgttccagatcctatagctggtgagcttccgggagctgttgttgtacttaagaaaggaaaatctatgactgaaaaagaagtaatggattacgttgctagtcaagtttcaaatgcaaaacgtttgcgtggtggtgtccgttttgtggacgaagtacctaaaggtctcactggtaaaattgacggtaaagcaattagagaaatactgaagaaaccagttgctaagatgtaa

SEQ ID NO: 4 - DNA, 30 bp, synthetic construct
  misc_feature 1..30: note = primer
  source 1..30: mol_type = other DNA
aatttctttagataaaggtgctccgccaga

SEQ ID NO: 5 - DNA, 30 bp, synthetic construct
  misc_feature 1..30: note = primer
  source 1..30: mol_type = other DNA
tctaaagaaattagcgaagctgttgctaga

SEQ ID NO: 6 - DNA, 30 bp, synthetic construct
  misc_feature 1..30: note = primer
  source 1..30: mol_type = other DNA
ttctccacgtctgttcgggcccaaagtttt

SEQ ID NO: 7 - DNA, 30 bp, synthetic construct
  misc_feature 1..30: note = primer
  source 1..30: mol_type = other DNA
agacgtggagaaattctggtaaagggtcct

SEQ ID NO: 8 - DNA, 30 bp, synthetic construct
  misc_feature 1..30: note = primer
  source 1..30: mol_type = other DNA
aatatttggatgttgcaaaagaacagattc

SEQ ID NO: 9 - DNA, 30 bp, synthetic construct
  misc_feature 1..30: note = primer
  source 1..30: mol_type = other DNA
catccaaatattattgatgccggcgttgct

SEQ ID NO: 10 - protein, 548 aa, Luciola lateralis
MENMENDENIVYGPEPFYPIEEGSAGAQLRKYMDRYAKLGAIAFTNALTGVDYTYAEYLEKSCCLGEALKNYGLVVDGRIALCSENCEEFFIPVLAGLFIGVGVAPTNEIYTLRELVHSLGISKPTIVFSSKKGLDKVITVQKTVTAIKTIVILDSKVDYRGYQSMDNFIKKNTPQGFKGSSFKTVEVNRKEQVALIMNSSGSTGLPKGVQLTHENLVTRFSHARDPIYGNQVSPGTAILTVVPFHHGFGMFTTLGYLTCGFRIVMLTKFDEETFLKTLQDYKCSSVILVPTLFAILNRSELLDKYDLSNLVEIASGGAPLSKEISEAVARRFNLPGVRQGYGLTETTSAIIITPEGDDKPGASGKVVPLFKAKVIDLDTKKTLGPNRRGEILVKGPMLMKGYVDNPEATREIIDEEGWLHTGDIGYYDEEKHFFIVDRLKSLIKYKGYQVPPAELESVLLQHPNIIDAGVAGVPDPIAGELPGAVVVLKKGKSMTEKEVMDYVASQVSNAKRLRGGVRFVDEVPKGLTGKIDGKAIREILKKPVAKM

SEQ ID NO: 11 - DNA, 1647 bp, Luciola lateralis
  source 1..1647: mol_type = other DNA
atggaaaacatggagaacgatgaaaatattgtgtatggtcctgaaccattttaccctattgaagagggatctgctggagcacaattgcgcaagtatatggatcgatatgcaaaacttggagcaattgcttttactaacgcacttaccggtgtcgattatacgtacgccgaatacttagaaaaatcatgctgtctaggagaggctttaaagaattatggtttggttgttgatggaagaattgcgttatgcagtgaaaactgtgaagagttctttattcctgtattagccggtttatttataggtgtcggtgtggctccaactaatgagatttacactctacgtgaattggttcacagtttaggcatctctaagccaacaattgtatttagttctaaaaaaggattagataaagttataactgtacaaaaaacggtaactgctattaaaaccattgttatattggacagcaaagtggattatagaggttatcaatccatggacaactttattaaaaaaaacactccacaaggtttcaaaggatcaagttttaaaactgtagaagttaaccgcaaagaacaagttgctcttataatgaactcttcgggttcaaccggtttgccaaaaggtgtgcaacttactcatgaaaatttggtcacgcgtttttctcacgctagagatccaatttatggaaaccaagtttcaccaggcacggctattttaactgtagtaccattccatcatggttttggtatgtttactactttaggctatctaacttgtggttttcgtattgtcatgttaacgaaatttgacgaagagacttttttaaaaacactgcaagattacaaatgttcaagcgttattcttgtaccgactttgtttgcaattcttaatagaagtgaattactcgataaatatgatttatcaaatttagttgaaattgcatctggcggagcacctttatctaaagaaattagcgaagctgttgctagacgttttaatttaccgggtgttcgtcaaggctatggtttaacagaaacaacctctgcaattattatcacaccggaaggcgatgataaaccaggtgcttctggcaaagttgtgccattatttaaagcaaaagttatcgatcttgatactaaaaaaactttgggcccgaacagacgtggagaaattctggtaaagggtcctatgcttatgaaaggttatgtagataatccagaagcaacaagagaaatcatagatgaagaaggttggttgcacacaggagatattgggtattacgatgaagaaaaacatttctttatcgtggatcgtttgaagtctttaatcaaatacaaaggatatcaagtaccacctgctgaattagaatctgttcttttgcaacatccaaatattattgatgccggcgttgctggcgttccagatcctatagctggtgagcttccgggagctgttgttgtacttaagaaaggaaaatctatgactgaaaaagaagtaatggattacgttgctagtcaagtttcaaatgcaaaacgtttgcgtggtggtgtccgttttgtggacgaagtacctaaaggtctcactggtaaaattgacggtaaagcaattagagaaatactgaagaaaccagttgctaagatgtaa

SEQ ID NO: 12 - DNA, 30 bp, synthetic construct
  misc_feature 1..30: note = primer
  source 1..30: mol_type = other DNA
ctcttcacagttttcactgcataacgcaat

SEQ ID NO: 13 - DNA, 30 bp, synthetic construct
  misc_feature 1..30: note = primer
  source 1..30: mol_type = other DNA
aactgtgaagagtactttattcctgtatta

SEQ ID NO: 14 - DNA, 30 bp, synthetic construct
  misc_feature 1..30: note = primer
  source 1..30: mol_type = other DNA
acgcgtgaccaaattctcgtgagtaagttg

SEQ ID NO: 15 - DNA, 30 bp, synthetic construct
  misc_feature 1..30: note = primer
  source 1..30: mol_type = other DNA
ttggtcacgcgtttatctcacgccagagat

SEQ ID NO: 16 - DNA, 30 bp, synthetic construct
  misc_feature 1..30: note = primer
  source 1..30: mol_type = other DNA
cataccaaaaccatggtgaaatgggactac

SEQ ID NO: 17 - DNA, 30 bp, synthetic construct
  misc_feature 1..30: note = primer
  source 1..30: mol_type = other DNA
ggttttggtatgttaactactttaggctat

SEQ ID NO: 18 - DNA, 30 bp, synthetic construct
  misc_feature 1..30: note = primer
  source 1..30: mol_type = other DNA
accacaagttagatagcctaaagtagtaaa

SEQ ID NO: 19 - DNA, 30 bp, synthetic construct
  misc_feature 1..30: note = primer
  source 1..30: mol_type = other DNA
ctaacttgtggttatcgtattgtcatgtta

SEQ ID NO: 20 - DNA, 30 bp, synthetic construct
  misc_feature 1..30: note = primer
  source 1..30: mol_type = other DNA
taatggcacaaccttaccagaagcacctgg

SEQ ID NO: 21 - DNA, 30 bp, synthetic construct
  misc_feature 1..30: note = primer
  source 1..30: mol_type = other DNA
gttgtgccattattgaaagcaaaagttatc

SEQ ID NO: 22 - DNA, 30 bp, synthetic construct
  misc_feature 1..30: note = primer
  source 1..30: mol_type = other DNA
caaagtcggtacaagaataacgcttgaaca

SEQ ID NO: 23 - DNA, 30 bp, synthetic construct
  misc_feature 1..30: note = primer
  source 1..30: mol_type = other DNA
gtaccgactttgctggcaattcttaataga

SEQ ID NO: 24 - DNA, 30 bp, synthetic construct
  misc_feature 1..30: note = primer
  source 1..30: mol_type = other DNA
accacaagttagatagcctaaagtagttaa

SEQ ID NO: 25 - DNA, 30 bp, synthetic construct
  misc_feature 1..30: note = primer
  source 1..30: mol_type = other DNA
tttcttcagtatttctctaattgctttacc

SEQ ID NO: 26 - DNA, 30 bp, synthetic construct
  misc_feature 1..30: note = primer
  source 1..30: mol_type = other DNA
taaggatccggctgctaacaaagcccgaaa

SEQ ID NO: 27 - protein, 543 aa, Luciola lateralis
MENMENDENIVYGPEPFYPIEEGSAGAQLRKYMDRYAKLGAIAFTNALTGVDYTYAEYLEKSCCLGEALKNYGLVVDGRIALCSENCEEFFIPVLAGLFIGVGVAPTNEIYTLRELVHSLGISKPTIVFSSKKGLDKVITVQKTVTAIKTIVILDSKVDYRGYQSMDNFIKKNTPQGFKGSSFKTVEVNRKEQVALIMNSSGSTGLPKGVQLTHENLVTRFSHARDPIYGNQVSPGTAILTVVPFHHGFGMLTTLGYLTCGYRIVMLTKFDEETFLKTLQDYKCSSVILVPTLLAILNRSELLDKYDLSNLVEIASGGAPLSKEIGEAVARRFNLPGVRQGYGLTETTSAIIITPEGDDKPGASGKVVPLFKAKVIDLDTKKTLGPNRRGEVLVKGPMLMKGYVDNPEATREIIDEEGWLHTGDIGYYDEEKHFFIVDRLKSLIKYKGYQVPPAELESVLLQHPNIFDAGVAGVPDPIAGELPGAVVVLKKGKSMTEKEVMDYVASQVSNAKRLRGGVRFVDEVPKGLTGKIDGKAIREILKK

SEQ ID NO: 28 - DNA, 1632 bp, Luciola lateralis
  source 1..1632: mol_type = other DNA
atggaaaacatggagaacgatgaaaatattgtgtatggtcctgaaccattttaccctattgaagagggatctgctggagcacaattgcgcaagtatatggatcgatatgcaaaacttggagcaattgcttttactaacgcacttaccggtgtcgattatacgtacgccgaatacttagaaaaatcatgctgtctaggagaggctttaaagaattatggtttggttgttgatggaagaattgcgttatgcagtgaaaactgtgaagagttctttattcctgtattagccggtttatttataggtgtcggtgtggctccaactaatgagatttacactctacgtgaattggttcacagtttaggcatctctaagccaacaattgtatttagttctaaaaaaggattagataaagttataactgtacaaaaaacggtaactgctattaaaaccattgttatattggacagcaaagtggattatagaggttatcaatccatggacaactttattaaaaaaaacactccacaaggtttcaaaggatcaagttttaaaactgtagaagttaaccgcaaagaacaagttgctcttataatgaactcttcgggttcaaccggtttgccaaaaggtgtgcaacttactcatgaaaatttggtcacgcgtttttctcacgctagagatccaatttatggaaaccaagtttcaccaggcacggctattttaactgtagtcccatttcaccatggttttggtatgttaactactttaggctatctaacttgtggttatcgtattgtcatgttaacgaaatttgacgaagagacttttttaaaaacactgcaagattacaaatgttcaagcgttattcttgtaccgactttgctggcaattcttaatagaagtgaattactcgataaatatgatttatcaaatttagttgaaattgcatctggcggagcacctttatctaaagaaattagcgaagctgttgctagacgttttaatttaccgggtgttcgtcaaggctatggtttaacagaaacaacctctgcaattattatcacaccggaaggcgatgataaaccaggtgcttctggcaaagttgtgccattatttaaagcaaaagttatcgatcttgatactaaaaaaactttgggcccgaacagacgtggagaaattctggtaaagggtcctatgcttatgaaaggttatgtagataatccagaagcaacaagagaaatcatagatgaagaaggttggttgcacacaggagatattgggtattacgatgaagaaaaacatttctttatcgtggatcgtttgaagtctttaatcaaatacaaaggatatcaagtaccacctgctgaattagaatctgttcttttgcaacatccaaatattattgatgccggcgttgctggcgttccagatcctatagctggtgagcttccgggagctgttgttgtacttaagaaaggaaaatctatgactgaaaaagaagtaatggattacgttgctagtcaagtttcaaatgcaaaacgtttgcgtggtggtgtccgttttgtggacgaagtacctaaaggtctcactggtaaaattgacggtaaagcaattagagaaatactgaagaaataa

SEQ ID NO: 29 - DNA, 30 bp, synthetic construct
  misc_feature 1..30: note = primer
  source 1..30: mol_type = other DNA
tggttcaggaccatacacaatattttcatc

SEQ ID NO: 30 - DNA, 30 bp, synthetic construct
  misc_feature 1..30: note = primer
  source 1..30: mol_type = other DNA
ggtcctgaaccagattaccctattgaagag

SEQ ID NO: 31 - DNA, 30 bp, synthetic construct
  misc_feature 1..30: note = primer
  source 1..30: mol_type = other DNA
ggtcctgaaccagaataccctattgaagag

SEQ ID NO: 32 - DNA, 30 bp, synthetic construct
  misc_feature 1..30: note = primer
  source 1..30: mol_type = other DNA
ggtcctgaaccaaagtaccctattgaagag

SEQ ID NO: 33 - DNA, 30 bp, synthetic construct
  misc_feature 1..30: note = primer
  source 1..30: mol_type = other DNA
aaatggttcaggaccatacacaatattttc

SEQ ID NO: 34 - DNA, 30 bp, synthetic construct
  misc_feature 1..30: note = primer
  source 1..30: mol_type = other DNA
cctgaaccatttttacctattgaagaggga

SEQ ID NO: 35 - DNA, 30 bp, synthetic construct
  misc_feature 1..30: note = primer
  source 1..30: mol_type = other DNA
tccaagttttgcatatcgatccatatactt

SEQ ID NO: 36 - DNA, 30 bp, synthetic construct
  misc_feature 1..30: note = primer
  source 1..30: mol_type = other DNA
gcaaaacttggagtaattgcttttactaac

SEQ ID NO: 37 - DNA, 30 bp, synthetic construct
  misc_feature 1..30: note = primer
  source 1..30: mol_type = other DNA
atcgacaccggtaagtgcgttagtaaaagc

SEQ ID NO: 38 - DNA, 30 bp, synthetic construct
  misc_feature 1..30: note = primer
  source 1..30: mol_type = other DNA
accggtgtcgatttaacgtacgccgaatac

SEQ ID NO: 39 - DNA, 30 bp, synthetic construct
  misc_feature 1..30: note = primer
  source 1..30: mol_type = other DNA
ctcattagttggagccacaccgacacctat

SEQ ID NO: 40 - DNA, 30 bp, synthetic construct
  misc_feature 1..30: note = primer
  source 1..30: mol_type = other DNA
ccaactaatgaggattacactctacgtgaa

SEQ ID NO: 41 - DNA, 30 bp, synthetic construct
  misc_feature 1..30: note = primer
  source 1..30: mol_type = other DNA
ccaactaatgaggaatacactctacgtgaa

SEQ ID NO: 42 - DNA, 30 bp, synthetic construct
  misc_feature 1..30: note = primer
  source 1..30: mol_type = other DNA
ccaactaatgagaagtacactctacgtgaa

SEQ ID NO: 43 - DNA, 30 bp, synthetic construct
  misc_feature 1..30: note = primer
  source 1..30: mol_type = other DNA
ccaactaatgagcgttacactctacgtgaa

SEQ ID NO: 44 - DNA, 30 bp, synthetic construct
  misc_feature 1..30: note = primer
  source 1..30: mol_type = other DNA
tttgctgtccaatataacaatggttttaat

SEQ ID NO: 45 - DNA, 30 bp, synthetic construct
  misc_feature 1..30: note = primer
  source 1..30: mol_type = other DNA
ttggacagcaaagatgattatagaggttat

SEQ ID NO: 46 - DNA, 30 bp, synthetic construct
  misc_feature 1..30: note = primer
  source 1..30: mol_type = other DNA
ttggacagcaaagaggattatagaggttat

SEQ ID NO: 47 - DNA, 30 bp, synthetic construct
  misc_feature 1..30: note = primer
  source 1..30: mol_type = other DNA
agaaaaacgcgtgaccaaattttcatgagt

SEQ ID NO: 48 - DNA, 30 bp, synthetic construct
  misc_feature 1..30: note = primer
  source 1..30: mol_type = other DNA
acgcgtttttctgtcgctagagatccaatt

SEQ ID NO: 49 - DNA, 30 bp, synthetic construct
  misc_feature 1..30: note = primer
  source 1..30: mol_type = other DNA
acgcgtttttctatcgctagagatccaatt

SEQ ID NO: 50 - DNA, 30 bp, synthetic construct
  misc_feature 1..30: note = primer
  source 1..30: mol_type = other DNA
acgcgtttttctctcgctagagatccaatt

SEQ ID NO: 51 - DNA, 30 bp, synthetic construct
  misc_feature 1..30: note = primer
  source 1..30: mol_type = other DNA
gtgagaaaaacgcgtgaccaaattttcatg

SEQ ID NO: 52 - DNA, 30 bp, synthetic construct
  misc_feature 1..30: note = primer
  source 1..30: mol_type = other DNA
cgtttttctcacattagagatccaatttat

SEQ ID NO: 53 - DNA, 30 bp, synthetic construct
  misc_feature 1..30: note = primer
  source 1..30: mol_type = other DNA
aattggatctctagcgtgagaaaaacgcgt

SEQ ID NO: 54 - DNA, 30 bp, synthetic construct
  misc_feature 1..30: note = primer
  source 1..30: mol_type = other DNA
agagatccaatttttggaaaccaagtttca

SEQ ID NO: 55 - DNA, 30 bp, synthetic construct
  misc_feature 1..30: note = primer
  source 1..30: mol_type = other DNA
agagatccaattttaggaaaccaagtttca

SEQ ID NO: 56 - DNA, 30 bp, synthetic construct
  misc_feature 1..30: note = primer
  source 1..30: mol_type = other DNA
gcctaaagtagttaacataccaaaaccatg

SEQ ID NO: 57 - DNA, 30 bp, synthetic construct
  misc_feature 1..30: note = primer
  source 1..30: mol_type = other DNA
actactttaggctttctaacttgtggttat

SEQ ID NO: 58 - DNA, 30 bp, synthetic construct
  misc_feature 1..30: note = primer
  source 1..30: mol_type = other DNA
tttatcgagtaattcacttctattaagaat

SEQ ID NO: 59 - DNA, 30 bp, synthetic construct
  misc_feature 1..30: note = primer
  source 1..30: mol_type = other DNA
ttactcgataaattcgatttatcaaattta

SEQ ID NO: 60 - DNA, 30 bp, synthetic construct
  misc_feature 1..30: note = primer
  source 1..30: mol_type = other DNA
taaatttgataaatcatatttatcgagtaa

SEQ ID NO: 61 - DNA, 30 bp, synthetic construct
  misc_feature 1..30: note = primer
  source 1..30: mol_type = other DNA
ttatcaaatttacgtgaaattgcatctggc

SEQ ID NO: 62 - DNA, 30 bp, synthetic construct
  misc_feature 1..30: note = primer
  source 1..30: mol_type = other DNA
ttatcaaatttagaagaaattgcatctggc

SEQ ID NO: 63 - DNA, 30 bp, synthetic construct
  misc_feature 1..30: note = primer
  source 1..30: mol_type = other DNA
ttatcaaatttaaaggaaattgcatctggc

SEQ ID NO: 64 - DNA, 30 bp, synthetic construct
  misc_feature 1..30: note = primer
  source 1..30: mol_type = other DNA
cccaatatctcctgtgtgcaaccaaccttc

SEQ ID NO: 65 - DNA, 30 bp, synthetic construct
  misc_feature 1..30: note = primer
  source 1..30: mol_type = other DNA
ggagatattgggttttacgatgaagaaaaa

SEQ ID NO: 66 - DNA, 30 bp, synthetic construct
  misc_feature 1..30: note = primer
  source 1..30: mol_type = other DNA
caaaccataattctttaaagcctctcctag

SEQ ID NO: 67 - DNA, 30 bp, synthetic construct
  misc_feature 1..30: note = primer
  source 1..30: mol_type = other DNA
aattatggtttgaaagttgatggaagaatt

SEQ ID NO: 68 - DNA, 30 bp, synthetic construct
  misc_feature 1..30: note = primer
  source 1..30: mol_type = other DNA
agagatccaatttatggaaaccaagtttca

SEQ ID NO: 69 - protein, 548 aa, Luciola cruciata [sequence omitted]

SEQ ID NO: 70 - DNA, 1647 bp, Luciola cruciata
  source 1..1647: mol_type = other DNA
atggaaaacatggaaaacgatgaaaatattgtagttggacctaaaccgttttaccctatcgaagagggatctgctggaacacaattacgcaaatacatggagcgatatgcaaaacttggcgcaattgcttttacaaatgcagttactggtgttgattattcttacgccgaatacttggagaaatcatgttgtctaggaaaagctttgcaaaattatggtttggttgttgatggcagaattgcgttatgcagtgaaaactgtgaagaattttttattcctgtaatagccggactgtttataggtgtaggtgttgcacccactaatgagatttacactttacgtgaactggttcacagtttaggtatctctaaaccaacaattgtatttagttctaaaaaaggcttagataaagttataacagtacagaaaacagtaactactattaaaaccattgttatactagatagcaaagttgattatcgaggatatcaatgtctggacacctttataaaaagaaacactccaccaggttttcaagcatccagtttcaaaactgtggaagttgaccgtaaagaacaagttgctcttataatgaactcttcgggttctaccggtttgccaaaaggcgtacaacttactcacgaaaatacagtcactagattttctcatgctagagatccgatttatggtaaccaagtttcaccaggcaccgctgttttaactgtcgttccattccatcatggttttggtatgttcactactctagggtatttaatttgtggttttcgtgttgtaatgttaacaaaattcgatgaagaaacatttttaaaaactctacaagattataaatgtacaagtgttattcttgtaccgaccttgtttgcaattctcaacaaaagtgaattactcaataaatacgatttgtcaaatttagttgagattgcatctggcggagcacctttatcaaaagaagttggtgaagctgttgctagacgctttaatcttcccggtgttcgtcaaggttatggtttaacagaaacaacatctgccattattattacaccagaaggagacgataaaccaggagcttctggaaaagtcgtgccgttgtttaaagcaaaagttattgatcttgataccaaaaaatctttaggtcctaacagacgtggagaagtttgtgttaaaggacctatgcttatgaaaggttatgtaaataatccagaagcaacaaaagaacttattgacgaagaaggttggctgcacaccggagatattggatattatgatgaagaaaaacatttctttattgtcgatcgtttgaagtctttaatcaaatacaaaggataccaagtaccacctgccgaattagaatccgttcttttgcaacatccatctatctttgatgctggtgttgccggcgttcctgatcctgtagctggcgagcttccaggagccgttgttgtactggaaagcggaaaaaatatgaccgaaaaagaagtaatggattatgttgcaagtcaagtttcaaatgcaaaacgtttacgtggtggtgttcgttttgtggatgaagtacctaaaggtcttactggaaaaattgacggcagagcaattagagaaatccttaagaaaccagttgctaagatgtga

SEQ ID NO: 71 - protein, 550 aa, Photinus pyralis
MEDAKNIKKGPAPFYPLEDGTAGEQLHKAMKRYALVPGTIAFTDAHIEVNITYAEYFEMSVRLAEAMKRYGLNTNHRIVVCSENSLQFFMPVLGALFIGVAVAPANDIYNERELLNSMNISQPTVVFVSKKGLQKILNVQKKLPIIQKIIIMDSKTDYQGFQSMYTFVTSHLPPGFNEYDFVPESFDRDKTIALIMNSSGSTGLPKGVALPHRTACVRFSHARDPIFGNQIIPDTAILSVVPFHHGFGMFTTLGYLICGFRVVLMYRFEEELFLRSLQDYKIQSALLVPTLFSFFAKSTLIDKYDLSNLHEIASGGAPLSKEVGEAVAKRFHLPGIRQGYGLTETTSAILITPEGDDKPGAVGKVVPFFEAKVVDLDTGKTLGVNQRGELCVRGPMIMSGYVNNPEATNALIDKDGWLHSGDIAYWDEDEHFFIVDRLKSLIKYKGYQVAPAELESILLQHPNIFDAGVAGLPDDDAGELPAAVVVLEHGKTMTEKEIVDYVASQVTTAKKLRGGVVFVDEVPKGLTGKLDARKIREILIKAKKGGKSKL

SEQ ID NO: 72 - DNA, 1653 bp, Photinus pyralis
  source 1..1653: mol_type = other DNA
atggaagacgccaaaaacataaagaaaggcccggcgccattctatccgctagaggatggaaccgctggagagcaactgcataaggctatgaagagatacgccctggttcctggaacaattgcttttacagatgcacatatcgaggtgaacatcacgtacgcggaatacttcgaaatgtccgttcggttggcagaagctatgaaacgatatgggctgaatacaaatcacagaatcgtcgtatgcagtgaaaactctcttcaattctttatgccggtgttgggcgcgttatttatcggagttgcagttgcgcccgcgaacgacatttataatgaacgtgaattgctcaacagtatgaacatttcgcagcctaccgtagtgtttgtttccaaaaaggggttgcaaaaaattttgaacgtgcaaaaaaaattaccaataatccagaaaattattatcatggattctaaaacggattaccagggatttcagtcgatgtacacgttcgtcacatctcatctacctcccggttttaatgaatacgattttgtaccagagtcctttgatcgtgacaaaacaattgcactgataatgaactcctctggatctactgggttacctaagggtgtggcccttccgcatagaactgcctgcgtcagattctcgcatgccagagatcctatttttggcaatcaaatcattccggatactgcgattttaagtgttgttccattccatcacggttttggaatgtttactacactcggatatttgatatgtggatttcgagtcgtcttaatgtatagatttgaagaagagctgtttttacgatcccttcaggattacaaaattcaaagtgcgttgctagtaccaaccctattttcattcttcgccaaaagcactctgattgacaaatacgatttatctaatttacacgaaattgcttctgggggcgcacctctttcgaaagaagtcggggaagcggttgcaaaacgcttccatcttccagggatacgacaaggatatgggctcactgagactacatcagctattctgattacacccgagggggatgataaaccgggcgcggtcggtaaagttgttccattttttgaagcgaaggttgtggatctggataccgggaaaacgctgggcgttaatcagagaggcgaattatgtgtcagaggacctatgattatgtccggttatgtaaacaatccggaagcgaccaacgccttgattgacaaggatggatggctacattctggagacatagcttactgggacgaagacgaacacttcttcatagttgaccgcttgaagtctttaattaaatacaaaggataccaggtggcccccgctgaattggagtcgatattgttacaacaccccaacatcttcgacgcgggcgtggcaggtcttcccgacgatgacgccggtgaacttcccgccgccgttgttgttttggagcacggaaagacgatgacggaaaaagagatcgtggattacgtcgccagtcaagtaacaaccgccaaaaagttgcgcggaggagttgtgtttgtggacgaagtaccgaaaggtcttaccggaaaactcgacgcaagaaaaatcagagagatcctcataaaggccaagaagggcggaaagtccaaattgtaa

SEQ ID NO: 73 - protein, 545 aa, Photuris pennsylvanica [sequence omitted]

SEQ ID NO: 74 - DNA, 1638 bp, Photuris pennsylvanica
  source 1..1638: mol_type = other DNA
atggaagataaaaatattttatatggacctgaaccatttcatcccttggctgatgggacggctggagaacagatgttttacgcattatctcggtatgcagatatttcaggatgcattgcattgacaaatgctcatacaaaagaaaatgttttatatgaagaatttttaaaattgtcgtgtcgtttagcggaaagttttaaaaagtatggattaaaacaaaacgacacaatagcggtgtgtagtgaaaatggtttgcaatttttccttcctttaattgcatcattgtatcttggaataattgcagcacctgttagtgataaatacattgaacgtgaattaatacacagtcttggtattgtaaaaccacgcataattttttgttccaagaatacttttcaaaaagtactgaatgtaaaatctaaattaaaatatgtagaaactattattatattagacttaaatgaagacttaggaggttatcaatgcctcaacaactttatttctcaaaattccgatattaatcttgacgtaaagaaatttaaaccaaattcttttaatcgagacgatcaggttgcgttggtaatgttttcttctggtacaactggtgtttctaagggagtcatgctaactcacaagaatattgttgcacgattttctcattgcaaagatcctacttttggtaacgcaattaatccaacgacagcaattttaacagtaataccattccaccatggttttggtatgactaccacattaggatactttacttgtggattccgagttgctctaatgcacacgtttgaagaaaaactatttttacaatcattacaagattataaagtggaaagtactttacttgtaccaacattaatggcattttttccaaaaagtgcgttagttgaaaagtacgatttatcgcacttaaaagaaattgcatctggtggcgcacctttatcaaaagaaattggggagatggtgaaaaaacggtttaaattaaactttgtcaggcaagggtatggattaacagaaaccacttcggctgttttaattacaccggacactgacgtcagaccgggatcaactggtaaaatagtaccatttcacgctgttaaagttgtggatcctacaacaggaaaaattttggggccaaatgaaactggagaattgtattttaaaggcgacatgataatgaaaagttattataataatgaagaagctactaaagcaattattaacaaagacggatggttgcgctctggtgatattgcttattatgacaatgatggccatttttatattgtggacaggctgaagtcattaattaaatataaaggttatcaggttgcacctgctgaaattgagggaatactcttacaacacccgtatattgttgatgccggcgttactggtataccggatgaagccgcgggcgagcttccagctgcaggtgttgtagtacagactggaaaatatctaaacgaacaaatcgtacaaaattttgtttccagtcaagtttcaacagccaaatggctacgtggtggggtgaaatttttggatgaaattcccaaaggatcaactggaaaaattgacagaaaagtgttaagacaaatgtttgaaaaacacaaatctaagctgtaa